European Patent Application EP 4 653 487 A1, published November 26, 2025. Title: METHOD FOR PRODUCING POLYMER COMPOUND. Applicant: Ｓｐｉｂｅｒ株式会社. Application JP. The sequence listing filed with the application follows.

SEQUENCE LISTING (9 sequences)

SEQ ID NO: 1 - protein, 2375 aa, synthetic construct
  source 1..2375: note = PRT799
MHHHHHHSSGSSGPGQQGPYGPGASAAAAAGQNGPGSGQQGPGQSGQYGPGQQGPGQQGPGSSAAAAAGPGQYGPGQQGPSASAAAAAGPGSGQQGPGASGQYGPGQQGPGQQGPGSSAAAAAGQYGSGPGQQGPYGSAAAAAGPGSGQYGQGPYGPGASGPGQYGPGQQGPSASAAAAAGSGQQGPGQYGPYASAAAAAGQYGSGPGQQGPYGPGQSGSGQQGPGQQGPYASAAAAAGPGQQGPYGPGSSAAAAAGQYGYGPGQQGPYGPGASGQNGPGSGQYGPGQQGPGQSAAAAAGPGQQGPYGPGASAAAAAGQYGPGQQGPGQYGPGSSGPGQQGPYGPGSSAAAAAGQYGPGQQGPYGPGQSAAAAAGQYQQGPGQQGPYGPGASGPGQQGPYGPGASAAAAAGPGQYGPGQQGPSASAAAAAGQYGSGPGQYGPYGPGQSGPGSGQQGQGPYGPGASAAAAAGQYGPGQQGPYGPGQSAAAAAGPGSGQYGPGASGQNGPGSGQYGPGQQGPGQSAAAAAGQYQQGPGQQGPYGPGASAAAAAGQYGSGPGQQGPYGPGQSGSGQQGPGQQGPYASAAAAAGPGSGQQGPGASGQQGPYGPGASAAAAAGQNGPGSGQQGPGQSGQYGPGQQGPGQQGPGSSAAAAAGPGQYGPGQQGPSASAAAAAGPGSGQQGPGASGQYGPGQQGPGQQGPGSSAAAAAGQYGSGPGQQGPYGSAAAAAGPGSGQYGQGPYGPGASGPGQYGPGQQGPSASAAAAAGSGQQGPGQYGPYASAAAAAGQYGSGPGQQGPYGPGQSGSGQQGPGQQGPYASAAAAAGPGQQGPYGPGSSAAAAAGQYGYGPGQQGPYGPGASGQNGPGSGQYGPGQQGPGQSAAAAAGPGQQGPYGPGASAAAAAGQYGPGQQGPGQYGPGSSGPGQQGPYGPGSSAAAAAGQYGPGQQGPYGPGQSAAAAAGQYQQGPGQQGPYGPGASGPGQQGPYGPGASAAAAAGPGQYGPGQQGPSASAAAAAGQYGSGPGQYGPYGPGQSGPGSGQQGQGPYGPGASAAAAAGQYGPGQQGPYGPGQSAAAAAGPGSGQYGPGASGQNGPGSGQYGPGQQGPGQSAAAAAGQYQQGPGQQGPYGPGASAAAAAGQYGSGPGQQGPYGPGQSGSGQQGPGQQGPYASAAAAAGPGSGQQGPGASGQQGPYGPGASAAAAAGQNGPGSGQQGPGQSGQYGPGQQGPGQQGPGSSAAAAAGPGQYGPGQQGPSASAAAAAGPGSGQQGPGASGQYGPGQQGPGQQGPGSSAAAAAGQYGSGPGQQGPYGSAAAAAGPGSGQYGQGPYGPGASGPGQYGPGQQGPSASAAAAAGSGQQGPGQYGPYASAAAAAGQYGSGPGQQGPYGPGQSGSGQQGPGQQGPYASAAAAAGPGQQGPYGPGSSAAAAAGQYGYGPGQQGPYGPGASGQNGPGSGQYGPGQQGPGQSAAAAAGPGQQGPYGPGASAAAAAGQYGPGQQGPGQYGPGSSGPGQQGPYGPGSSAAAAAGQYGPGQQGPYGPGQSAAAAAGQYQQGPGQQGPYGPGASGPGQQGPYGPGASAAAAAGPGQYGPGQQGPSASAAAAAGQYGSGPGQYGPYGPGQSGPGSGQQGQGPYGPGASAAAAAGQYGPGQQGPYGPGQSAAAAAGPGSGQYGPGASGQNGPGSGQYGPGQQGPGQSAAAAAGQYQQGPGQQGPYGPGASAAAAAGQYGSGPGQQGPYGPGQSGSGQQGPGQQGPYASAAAAAGPGSGQQGPGASGQQGPYGPGASAAAAAGQNGPGSGQQGPGQSGQYGPGQQGPGQQGPGSSAAAAAGPGQYGPGQQGPSASAAAAAGPGSGQQGPGASGQYGPGQQGPGQQGPGSSAAAAAGQYGSGPGQQGPYGSAAAAAGPGSGQYGQGPYGPGASGPGQYGPGQQGPSASAAAAAGSGQQGPGQYGPYASAAAAAGQYGSGPGQQGPYGPGQSGSGQQGPGQQGPYASAAAAAGPGQQGPYGPGSSAAAAAGQYGYGPGQQGPYGPGASGQNGPGSGQYGPGQQGPGQSAAAAAGPGQQGPYGPGASAAAAAGQYGPGQQGPGQYGPGSSGPGQQGPYGPGSSAAAAAGQYGPGQQGPYGPGQSAAAAAGQYQQGPGQQGPYGPGASGPGQQGPYGPGASAAAAAGPGQYGPGQQGPSASAAAAAGQYGSGPGQYGPYGPGQSGPGSGQQGQGPYGPGASAAAAAGQYGPGQQGPYGPGQSAAAAAGPGSGQYGPGASGQNGPGSGQYGPGQQGPGQSAAAAAGQYQQGPGQQGPYGPGASAAAAAGQYGSGPGQQGPYGPGQSGSGQQGPGQQGPYASAAAAAGPGSGQQGSSVDKLAAALEHHHHHH

SEQ ID NO: 2 - protein, 1190 aa, synthetic construct
  source 1..1190: note = PRT966
MHHHHHHSSGSSGPGVFGPYGPGASAAAAAGINGPGSGVFGPGISGIYGPGVFGPGVFGPGSSAAAAAGPGIYGPGVFGPSASAAAAAGPGSGVFGPGASGIYGPGVFGPGVFGPGSSAAAAAGIYGSGPGVFGPYGSAAAAAGPGSGIYGIGPYGPGASGPGIYGPGVFGPSASAAAAAGSGVFGPGIYGPYASAAAAAGIYGSGPGVFGPYGPGISGSGVFGPGVFGPYASAAAAAGPGVFGPYGPGSSAAAAAGIYGYGPGVFGPYGPGASGINGPGSGIYGPGVFGPGISAAAAAGPGVFGPYGPGASAAAAAGIYGPGVFGPGIYGPGSSGPGVFGPYGPGSSAAAAAGIYGPGVFGPYGPGISAAAAAGIYVFGPGVFGPYGPGASGPGVFGPYGPGASAAAAAGPGIYGPGVFGPSASAAAAAGIYGSGPGIYGPYGPGISGPGSGVFGIGPYGPGASAAAAAGIYGPGVFGPYGPGISAAAAAGPGSGIYGPGASGINGPGSGIYGPGVFGPGISAAAAAGIYVFGPGVFGPYGPGASAAAAAGIYGSGPGVFGPYGPGISGSGVFGPGVFGPYASAAAAAGPGSGVFGPGASGPGVFGPYGPGASAAAAAGINGPGSGVFGPGISGIYGPGVFGPGVFGPGSSAAAAAGPGIYGPGVFGPSASAAAAAGPGSGVFGPGASGIYGPGVFGPGVFGPGSSAAAAAGIYGSGPGVFGPYGSAAAAAGPGSGIYGIGPYGPGASGPGIYGPGVFGPSASAAAAAGSGVFGPGIYGPYASAAAAAGIYGSGPGVFGPYGPGISGSGVFGPGVFGPYASAAAAAGPGVFGPYGPGSSAAAAAGIYGYGPGVFGPYGPGASGINGPGSGIYGPGVFGPGISAAAAAGPGVFGPYGPGASAAAAAGIYGPGVFGPGIYGPGSSGPGVFGPYGPGSSAAAAAGIYGPGVFGPYGPGISAAAAAGIYVFGPGVFGPYGPGASGPGVFGPYGPGASAAAAAGPGIYGPGVFGPSASAAAAAGIYGSGPGIYGPYGPGISGPGSGVFGIGPYGPGASAAAAAGIYGPGVFGPYGPGISAAAAAGPGSGIYGPGASGINGPGSGIYGPGVFGPGISAAAAAGIYVFGPGVFGPYGPGASAAAAAGIYGSGPGVFGPYGPGISGSGVFGPGVFGPYASAAAAAGPGSGVFGPGAS

SEQ ID NO: 3 - protein, 601 aa, synthetic construct
  source 1..601: note = PRT918
MHHHHHHSSGSSGPGVFGPYGPGASAAAAAGINGPGSGVFGPGISGIYGPGVFGPGVFGPGSSAAAAAGPGIYGPGVFGPSASAAAAAGPGSGVFGPGASGIYGPGVFGPGVFGPGSSAAAAAGIYGSGPGVFGPYGSAAAAAGPGSGIYGIGPYGPGASGPGIYGPGVFGPSASAAAAAGSGVFGPGIYGPYASAAAAAGIYGSGPGVFGPYGPGISGSGVFGPGVFGPYASAAAAAGPGVFGPYGPGSSAAAAAGIYGYGPGVFGPYGPGASGINGPGSGIYGPGVFGPGISAAAAAGPGVFGPYGPGASAAAAAGIYGPGVFGPGIYGPGSSGPGVFGPYGPGSSAAAAAGIYGPGVFGPYGPGISAAAAAGIYVFGPGVFGPYGPGASGPGVFGPYGPGASAAAAAGPGIYGPGVFGPSASAAAAAGIYGSGPGIYGPYGPGISGPGSGVFGIGPYGPGASAAAAAGIYGPGVFGPYGPGISAAAAAGPGSGIYGPGASGINGPGSGIYGPGVFGPGISAAAAAGIYVFGPGVFGPYGPGASAAAAAGIYGSGPGVFGPYGPGISGSGVFGPGVFGPYASAAAAAGPGSGVFGPGAS

SEQ ID NO: 4 - protein, 608 aa, synthetic construct
  source 1..608: note = PRT313
MHHHHHHSSGSSGPGGQGPYGPGASAAAAAGGNGPGSGQQGPGGSAAAAAGGYGPGGQGPGQQGPGSSAAAAAGPGGYGPGGQGPSASAAAAAGPGSGQQGPGASAAAAAGGYGPGGQGPGQQGPGSSAAAAAGGYGSGPGQQGPYGSAAAAAGPGSGGYGQGPYGPGASAAAAAGPGGYGPGGQGPSASAAAAAGSGQQGPGGYGPYASAAAAAGGYGSGPGQQGPYGPGGSAAAAAGSGQQGPGQQGPYASAAAAAGPGGQGPYGPGSSAAAAAGGYGYGPGGQGPYGPGASAAAAAGGNGPGSGGYGPGQQGPGGSAAAAAGPGGQGPYGPGASAAAAAGGYGPGGQGPGGYGPGSSAAAAAGPGGQGPYGPGSSAAAAAGGYGPGQQGPYGPGGSAAAAAGGYQQGPGGQGPYGPGASAAAAAGPGGQGPYGPGASAAAAAGPGGYGPGGQGPSASAAAAAGGYGSGPGGYGPYGPGGSAAAAAGPGSGQQGQGPYGPGASAAAAAGGYGPGQQGPYGPGGSAAAAAGPGSGGYGPGASAAAAAGGNGPGSGGYGPGQQGPGGSAAAAAGGYQQGPGGQGPYGPGASAAAAAGPGSGQQGPGAS

SEQ ID NO: 5 - protein, 603 aa, synthetic construct
  source 1..603: note = PRT1000
MHHHHHHSSGSSCGPGVFGPYGPGASAAAAAGINGPGSGVFGPGISGIYGPGVFGPGVFGPGSSAAAAAGPGIYGPGVFGPSASAAAAAGPGSGVFGPGASGIYGPGVFGPGVFGPGSSAAAAAGIYGSGPGVFGPYGSAAAAAGPGSGIYGIGPYGPGASGPGIYGPGVFGPSASAAAAAGSGVFGPGIYGPYASAAAAAGIYGSGPGVFGPYGPGISGSGVFGPGVFGPYASAAAAAGPGVFGPYGPGSSAAAAAGIYGYGPGVFGPYGPGASGINGPGSGIYGPGVFGPGISAAAAAGPGVFGPYGPGASAAAAAGIYGPGVFGPGIYGPGSSGPGVFGPYGPGSSAAAAAGIYGPGVFGPYGPGISAAAAAGIYVFGPGVFGPYGPGASGPGVFGPYGPGASAAAAAGPGIYGPGVFGPSASAAAAAGIYGSGPGIYGPYGPGISGPGSGVFGIGPYGPGASAAAAAGIYGPGVFGPYGPGISAAAAAGPGSGIYGPGASGINGPGSGIYGPGVFGPGISAAAAAGIYVFGPGVFGPYGPGASAAAAAGIYGSGPGVFGPYGPGISGSGVFGPGVFGPYASAAAAAGPGCSGVFGPGAS

SEQ ID NO: 6 - protein, 605 aa, synthetic construct
  source 1..605: note = PRT1001
MHHHHHHSSGSSCGPGVFGPYGPGASAAAAAGINGPGSGVFGPGISCGIYGPGVFGPGVFGPGSSAAAAAGPGIYGPGVFGPSASAAAAAGPGSGVFGPGASGIYGPGVFGPGVFGPGSSAAAAAGIYGSGPGVFGPYGSAAAAAGPGSGIYGIGPYGPGASGPGIYGPGVFGPSASAAAAAGSGVFGPGIYGPYASAAAAAGIYGSGPGVFGPYGPGISGSGVFGPGVFGPYASAAAAAGPGVFGPYGPGSSAAAAAGIYGYGPGVFGPYGPGASGINGPGSGIYGPGVFGPGISAAAAAGPGVFGPYGPGASAAAAAGIYGPGVFGPGIYGPGSSGPGVFGPYGPGSSAAAAAGIYGPGVFGPYGPGISAAAAAGIYVFGPGVFGPYGPGASGPGVFGPYGPGASAAAAAGPGIYGPGVFGPSASAAAAAGIYGSGPGIYGPYGPGISGPGSGVFGIGPYGPGASAAAAAGIYGPGVFGPYGPGISAAAAAGPGSGIYGPGASGINGPGSGIYGPGVFGPGISAAAAAGIYVFGPGVFGPYGPGASAAAAAGIYGSGPGVFGPYGPGISGCSGVFGPGVFGPYASAAAAAGPGCSGVFGPGAS

SEQ ID NO: 7 - protein, 1188 aa, synthetic construct
  source 1..1188: note = PRT587
MHHHHHHSSGSSGPGQQGPYGPGASAAAAAGQNGPGSGQQGPGQSGQYGPGQQGPGQQGPGSSAAAAAGPGQYGPGQQGPSASAAAAAGPGSGQQGPGASGQYGPGQQGPGQQGPGSSAAAAAGQYGSGPGQQGPYGSAAAAAGPGSGQYGQGPYGPGASGPGQYGPGQQGPSASAAAAAGSGQQGPGQYGPYASAAAAAGQYGSGPGQQGPYGPGQSGSGQQGPGQQGPYASAAAAAGPGQQGPYGPGSSAAAAAGQYGYGPGQQGPYGPGASGQNGPGSGQYGPGQQGPGQSAAAAAGPGQQGPYGPGASAAAAAGQYGPGQQGPGQYGPGSSGPGQQGPYGPGSSAAAAAGQYGPGQQGPYGPGQSAAAAAGQYQQGPGQQGPYGPGASGPGQQGPYGPGASAAAAAGPGQYGPGQQGPSASAAAAAGQYGSGPGQYGPYGPGQSGPGSGQQGQGPYGPGASAAAAAGQYGPGQQGPYGPGQSAAAAAGPGSGQYGPGASGQNGPGSGQYGPGQQGPGQSAAAAAGQYQQGPGQQGPYGPGASAAAAAGQYGSGPGQQGPYGPGQSGSGQQGPGQQGPYASAAAAAGPGSGQQGPGASGQQGPYGPGASAAAAAGQNGPGSGQQGPGQSGQYGPGQQGPGQQGPGSSAAAAAGPGQYGPGQQGPSASAAAAAGPGSGQQGPGASGQYGPGQQGPGQQGPGSSAAAAAGQYGSGPGQQGPYGSAAAAAGPGSGQYGQGPYGPGASGPGQYGPGQQGPSASAAAAAGSGQQGPGQYGPYASAAAAAGQYGSGPGQQGPYGPGQSGSGQQGPGQQGPYASAAAAAGPGQQGPYGPGSSAAAAAGQYGYGPGQQGPYGPGASGQNGPGSGQYGPGQQGPGQSAAAAAGPGQQGPYGPGASAAAAAGQYGPGQQGPGQYGPGSSGPGQQGPYGPGSSAAAAAGQYGPGQQGPYGPGQSAAAAAGQYQQGPGQQGPYGPGASGPGQQGPYGPGASAAAAAGPGQYGPGQQGPSASAAAAAGQYGSGPGQYGPYGPGQSGPGSGQQGQGPYGPGASAAAAAGQYGPGQQGPYGPGQSAAAAAGPGSGQYGPGASGQNGPGSGQYGPGQQGPGQSAAAAAGQYQQGPGQQGPYGPGASAAAAAGQYGSGPGQQGPYGPGQSGSGQQGPGQQGPYASAAAAAGPGSGQQGPGAS

SEQ ID NO: 8 - protein, 24 aa, synthetic construct
  source 1..24: note = His tag and Hindge sequence
MHHHHHHHHHHSSGSSLEVLFQGP

SEQ ID NO: 9 - protein, 110 aa, synthetic construct
  source 1..110: note = PRT2882
MHHHHHHSSGSSCGPGVFGPYGPGASAAAAAGINGPGSGVFGPGISGIYGPGVFGPGVFGPGSSAAAAAGPGIYGPGVFGPSASAAAAAGPGCSGVFGPGASGFILGFIL